European Patent Application EP 4 516 912 A1, published March 5, 2025. Title: HERBICIDE RESISTANT PLANTS. Applicant: Eberhard-Karls-Universität Tübingen. Application EP. The sequence listing filed with the application follows.

SEQUENCE LISTING (7 sequences)

SEQ ID NO: 1 - protein, 442 aa, Arabidopsis thaliana
MAANTISLSNVAASKNLNSFQSRAFIAPPTIFFPVASAKSKPGELSLSSTTLSRSRVRAGASQLMNEPLNDQRSISSPTVVEVDLGDRSYPIYIGAGLLDHSELLQRHVHGKRVLVVTNDRVAPLYLDKTIDALTRGNPNVTVESVILPDGEKYKDMDTLMKVFDKAIESRLDRRCTFVALGGGVIGDMCGYAAASYLRGVNFIQIPTTVMAQVDSSVGGKTGINHRLGKNLIGAFYQPQCVLVDTDTLNTLPDREMASGLAEVIKYGLIRDAEFFEWQEKNIEALLARDPAALAFAIKRSCENKADVVSQDEKESGLRATLNLGHTFGHAIETGFGYGEWLHGEAVAAGTVMAVDMSYRLGWIDESIVKRVNKILVRAKLPTTPPESMTVSMFKSIMAVDKKVADGLLRLILLKGPLGNCVFTGDYDREALDATLRAFSKS

SEQ ID NO: 2 - protein, 444 aa, Brassica nappus
MALPLVSSVSYIKSSNQFHCSFSLRKEKFELSSFFIVLCSHFSYVDTAERLELDRLLLWSSHQKIRFSKRTFSQRIVVKMSASTLPMNLGKAKKVWIWTMCKEVMTVAVERGWNTFIFSSDNRKLSNEWSSIALMDTLFIEEKKVIDGTGNVVASVFEVSTPEELRSLNIENEQIENIVLDFLDWKSIPAENLVAALQGSEKTVFAVSNTPSEAKLFLEALEHGLGGIILKSEDVKAVLDLKEYFDKRNEESDTLSLTEATITRVQMVGMGDRVCVDLCSLMRPGEGLLVGSFARGLFLVHSECLESNYIESRPFRVNAGPVHAYVAVPGGKTCYLSELRTGREVIVVDQKGKQRTAVVGRVKIEKRPLIVVEAKLSTKEEETVYSIILQNAETVALVTPHQVNSSGRTAVPVTSLKPGDQVLIRLQGGARHTGIEIQEFIVEN

SEQ ID NO: 3 - protein, 440 aa, Brassica rapa
MAANAVSLSISSTVASSKTLHSLQAQTRGLIPPPTISFPKSSSSLSSTTISISRSRVRAGPSQLVNEPANAMATPPTIVEVDLGSRSYPIYIGAGLLDQSHLLQRHVHGKKVLVVTNERVAPLYLDKTVHALTIGNPNVTVESVILPDGEKYKDMDTLMKVFDKAIESRLDRRSTFVALGGGVIGDMCGYAAASYLRGVNFIQIPTTVMAQVDSSVGGKTGINHRLGKNLIGAFYQPQCVLVDTDTLNTLPDREMASGLAEVIKYGLIRDADFFEWQEKNIEALLARDPAALAYAIKRSCENKADVVSQDEKESGLRATLNLGHTFGHAIETGFGYGEWLHGEAVAAGTVMAVDMSHRLGWIDDSIVERVNNILKRAKLPTTPPESMTVSMFKSIMAVDKKVADGLLRLILLKGPLGNCVFTGDYDREALDATLRAFSKS

SEQ ID NO: 4 - protein, 463 aa, Hordeum vulgare
LIGGNRTQPPPPPPPFRDQTTPMAASASSLLAAAASSSSRAAISVRRPRAAPAAAAASVPSSSRSSFTPLRASPARALRSRVVASAAPAMQPPAVSRVSTVVDVDLGDRSYPIYIGPGLLNEPDLLQRHVIGKRVLVVTNTTVAPLYLEKVTWALTHQNPNVSVESVILPDGEKYKDMDTLMKVFDKAVESRLDRRCTFVALGGGVIGDMCGFAASAFLRGVNFIQIPTTLMAQVDSSVGGKTGINHPLGKNLIGAFYQPQCVLIDTETLNTLPDRELASGVAEVVKYGLIRDAPFFEWQEKNMAAILAREPSALTYAIKRSCENKAEVVAQDEKESGLRATLNLGHTFGHAIETGLGYGEWLHGEAVAAGTVMAADMSYRLGWIDESIKKRTFDILDQAKLPVTPPKGMTVEKFRNIMAVDKKVADGLLRLILLKGPLGGCVFTGEYDRKALDETLRAFCDE

SEQ ID NO: 5 - protein, 444 aa, Arabidopsis thaliana; identical to SEQ ID NO: 2

SEQ ID NO: 6 - protein, 425 aa, Brassica rapa
MALPLVSSVSYIQSSSTQLHCFPLRKERFGLYRLQTWSSHHSSTRLIRKKTFPQRLAVRMSASSTLPMNLQRSKKVWIWTECKEVMTTAVERGWNTFVFSSDSLQLSDDWSSVALVDALFIDERQVTDGTGRVVAAVFEVSTPEELQMLKIENEQAENIVLGLLDWKSIPAENLVAALQGSEKTVFAISSTPSEAKLYLEALEHGLGGIILKTEDVKAVLDLKEYFDKRGEESDTLSLTEATITRIEMVGMGDRVCVDLCSLMRPGEGLLVGSFARGLFLVHSECLESNYIASRPFRVNAGPVHAYVAVPGGRTCYLSELRTGRQVIVVDQKGKQRTAVVGRVKIEKRPLILVEAKLSGEEDETSFSTILQNAETVALVTPHQVNSSGKTAVPVTSLKLGDQVLIRLQGGARHTGIEIQEFIVEN

SEQ ID NO: 7 - protein, 420 aa, Hordeum vulgare
KTGANDQMPHPEIPQRNSMAVSCSSSSSSILGSAKSLACFHTSNLAPQRTASARSRLQSIKMRSAPAAPGESKKTVWVWTENRQVMTAAVERGWNTFLFGSKDVGKDWSSTARIHPLFIDGLEIFDEGNQKVATISEISSPSELQLIQPDNVEVQNTVIHFRGDWQVIPAENIVAAFQGCAGTVLAVSTNSTEAQVFLEALEQGLNGVVLKVEDMDDIIKLKDYFDRRNEAKSQLQLTKATVSKVEVVGMGDRVCVDLCSIMRPGEGLLVGSYARGMFLVHSECLETNYIASRPFRVNAGPVHAYVTVPGDKTSYLSELQSGREVIVVDQNGLWRTSIVGRVKIESRPLILVEAKENSGNGTYSIFLQNAETVALIGPDRGSGGRTAIPVTSLKVGDEVLVRKQGGARHTGIEIQEFIVE